European Patent Application EP 4 194 555 A1, published June 14, 2023. Title: DNA aptamers inhibiting binding of Urokinase type plasminogen activator (uPA) with Urokinase type plasminogen activator receptor (uPAR) and inhibiting uPA activity. Applicant: Fraunhofer-Gesellschaft zur Förderung der angewandten Forschung e.V. The sequence listing filed with the application follows.

SEQUENCE LISTING (25 sequences)

SEQ ID NO: 1 - DNA, 82 bp, artificial sequence
  uPAapt-01
aggtagaggagcaagccatcatggtaacatgcactaggtcgcgatggttccgtctgatcgctgatgcgtgatcgaacctacc

SEQ ID NO: 2 - DNA, 82 bp, artificial sequence
  uPAapt-02
aggtagaggagcaagccatccaagcgggggtgagagatctgtcagtacgagctgggtttgcggatgcgtgatcgaacctacc

SEQ ID NO: 3 - DNA, 62 bp, artificial sequence
  uPAapt-02-R
aggtagaggagcaagccatccaagcgggggtgagagatctgtcagtacgagctgggtttgcg

SEQ ID NO: 4 - DNA, 62 bp, artificial sequence
  uPAapt-02-F
caagcgggggtgagagatctgtcagtacgagctgggtttgcggatgcgtgatcgaacctacc

SEQ ID NO: 5 - DNA, 42 bp, artificial sequence
  uPAapt-02-FR
caagcgggggtgagagatctgtcagtacgagctgggtttgcg

SEQ ID NO: 6 - DNA, 82 bp, artificial sequence
  uPAapt-03
aggtagaggagcaagccatcacggaggcagagggtgagagatctgttagtactagcccatgtgatgcgtgatcgaacctacc

SEQ ID NO: 7 - DNA, 82 bp, artificial sequence
  uPAapt-06
aggtagaggagcaagccatcgggtgggtgggtgggtgatggctcgactctaccctggcgctggatgcgtgatcgaacctacc

SEQ ID NO: 8 - DNA, 81 bp, artificial sequence
  uPAapt-08
aggtagaggagcaagccatccagcggtaggggttatatagctgcgccatagggtactcgtggatgcgtgatcgaacctacc

SEQ ID NO: 9 - DNA, 82 bp, artificial sequence
  uPAapt-21
aggtagaggagcaagccatcggaggtactcaccgacgctgaactccatagaatgtggtgatggatgcgtgatcgaacctacc

SEQ ID NO: 10 - DNA, 82 bp, artificial sequence
  uPAapt-26
aggtagaggagcaagccatcatccgtggcgtggttggtgggggaggtgggcgggtagacggtgatgcgtgatcgaacctacc

SEQ ID NO: 11 - DNA, 82 bp, artificial sequence
  uPAapt-27
aggtagaggagcaagccatcatggggtgttatggggggggcttattgcggtcaggggacgatgatgcgtgatcgaacctacc

SEQ ID NO: 12 - DNA, 42 bp, artificial sequence
  uPAapt-01-FR
atggtaacatgcactaggtcgcgatggttccgtctgatcgct

SEQ ID NO: 13 - DNA, 41 bp, artificial sequence
  uPAapt-08-FR
cagcggtaggggttatatagctgcgccatagggtactcgtg

SEQ ID NO: 14 - DNA, 62 bp, artificial sequence
  uPAapt-27-F
atggggtgttatggggggggcttattgcggtcaggggacgatgatgcgtgatcgaacctacc

SEQ ID NO: 15 - DNA, 62 bp, artificial sequence
  uPAapt-27-R
aggtagaggagcaagccatcatggggtgttatggggggggcttattgcggtcaggggacgat

SEQ ID NO: 16 - DNA, 42 bp, artificial sequence
  uPAapt-27-FR
atggggtgttatggggggggcttattgcggtcaggggacgat

SEQ ID NO: 17 - DNA, 20 bp, artificial sequence
  forward primer [5'-Primer]
aggtagaggagcaagccatc

SEQ ID NO: 18 - DNA, 20 bp, artificial sequence
  reverse primer binding site [3'-Primer of forward strain]
gatgcgtgatcgaacctacc

SEQ ID NO: 19 - protein, 411 aa, artificial sequence
  pro-uPA
SNELHQVPSNCDCLNGGTCVSNKYFSNIHWCNCPKKFGGQHCEIDKSKTCYEGNGHFYRGKASTDTMGRPCLPWNSATVLQQTYHAHRSDALQLGLGKHNYCRNPDNRRRPWCYVQVGLKPLVQECMVHDCADGKKPSSPPEELKFQCGQKTLRPRFKIIGGEFTTIENQPWFAAIYRRHRGGSVTYVCGGSLISPCWVISATHCFIDYPKKEDYIVYLGRSRLNSNTQGEMKFEVENLILHKDYSADTLAHHNDIALLKIRSKEGRCAQPSRTIQTICLPSMYNDPQFGTSCEITGFGKENSTDYLYPEQLKMTVVKLISHRECQQPHYYGSEVTTKMLCAADPQWKTDSCQGDSGGPLVCSLQGRMTLTGIVSWGRGCALKDKPGVYTRVSHFLPWIRSHTKEENGLAL

SEQ ID NO: 20 - protein, 158 aa, artificial sequence
  HMW-uPA - A Chain
SNELHQVPSNCDCLNGGTCVSNKYFSNIHWCNCPKKFGGQHCEIDKSKTCYEGNGHFYRGKASTDTMGRPCLPWNSATVLQQTYHAHRSDALQLGLGKHNYCRNPDNRRRPWCYVQVGLKPLVQECMVHDCADGKKPSSPPEELKFQCGQKTLRPRFK

SEQ ID NO: 21 - protein, 253 aa, artificial sequence
  HMW-uPA - B Chain
IIGGEFTTIENQPWFAAIYRRHRGGSVTYVCGGSLISPCWVISATHCFIDYPKKEDYIVYLGRSRLNSNTQGEMKFEVENLILHKDYSADTLAHHNDIALLKIRSKEGRCAQPSRTIQTICLPSMYNDPQFGTSCEITGFGKENSTDYLYPEQLKMTVVKLISHRECQQPHYYGSEVTTKMLCAADPQWKTDSCQGDSGGPLVCSLQGRMTLTGIVSWGRGCALKDKPGVYTRVSHFLPWIRSHTKEENGLAL

SEQ ID NO: 22 - protein, 23 aa, artificial sequence
  LMW-uPA - (Residue) A Chain
KPSSPPEELKFQCGQKTLRPRFK

SEQ ID NO: 23 - protein, 253 aa, artificial sequence; identical to SEQ ID NO: 21
  LMW-uPA - B Chain

SEQ ID NO: 24 - DNA, 79 bp, artificial sequence
  Con - sequence-unrelated control aptamer
gggaattcgagctcggtaccgtacagtactgcatatctcatacttcctagataccatccctgcaggcatgcaagcttgg

SEQ ID NO: 25 - DNA, 20 bp, artificial sequence
  Reverse primer
ggtaggttcgatcacgcatc